European Patent Application EP 4 223 873 A2, published August 9, 2023. Title: COMPOSITIONS AND METHODS FOR T CELL DELIVERY OF THERAPEUTIC MOLECULES. Applicant: The Trustees of the University of Pennsylvania. Application EP, filed October 30, 2015. The sequence listing filed with the application follows.

SEQUENCE LISTING (18 sequences)

SEQ ID NO: 1 - DNA, 717 bp, Homo sapiens
  source 1..717: mol_type = other DNA
atggaggcggcggtcgctgctccgcgtccccggctgctcctcctcgtgctggcggcggcggcggcggcggcggcggcgctgctcccgggggcgacggcgttacagtgtttctgccacctctgtacaaaagacaattttacttgtgtgacagatgggctctgctttgtctctgtcacagagaccacagacaaagttatacacaacagcatgtgtatagctgaaattgacttaattcctcgagataggccgtttgtatgtgcaccctcttcaaaaactgggtctgtgactacaacatattgctgcaatcaggaccattgcaataaaatagaacttccaactactgtaaagtcatcacctggccttggtcctgtggaactggcagctgtcattgctggaccagtgtgcttcgtctgcatctcactcatgttgatggtctatatcagggccgcacggcacctgtgcccgccgctgcccacaccctgtgccagctccgccattgagttccctggagggaaggagacttggcagtggatcaacccagtggacttccaggaagaggcatccctgcaggaggccctggtggtagagatgtcctgggacaaaggcgagaggactgagcctctcgagaagacagagctacctgagggtgcccctgagctggccctggatacagagttgtccttggaggatggagacaggtgcaaggccaagatgtga

SEQ ID NO: 2 - DNA, 1212 bp, Homo sapiens
  source 1..1212: mol_type = other DNA
atgggtcgggggctgctcaggggcctgtggccgctgcacatcgtcctgtggacgcgtatcgccagcacgatcccaccgcacgttcagaagtcggttaataacgacatgatagtcactgacaacaacggtgcagtcaagtttccacaactgtgtaaattttgtgatgtgagattttccacctgtgacaaccagaaatcctgcatgagcaactgcagcatcacctccatctgtgagaagccacaggaagtctgtgtggctgtatggagaaagaatgacgagaacataacactagagacagtttgccatgaccccaagctcccctaccatgactttattctggaagatgctgcttctccaaagtgcattatgaaggaaaaaaaaaagcctggtgagactttcttcatgtgttcctgtagctctgatgagtgcaatgacaacatcatcttctcagaagaatataacaccagcaatcctgacttgttgctagtcatatttcaagtgacaggcatcagcctcctgccaccactgggagttgccatatctgtcatcatcatcttctaccagcaaaaggtgtttgttctcctagcagccctcagacctcagtggtgtagcagagaaattccagatccagcaaatagcacttgcgctaagaaatatcccattgcagaggagaagacacagctgcccttggacaggctcctgatagactggcccacgcctgaagatcctgaaccgctggtcatcagtgaagtccttcatcaagtgaccccagttttcagacatcccccctgctccaactggccacaaagggaaaaaggaatccaaggtcatcaggcctctgagaaagacatgatgcacagtgcctcaagcccaccacctccaagagctctccaagctgagagcagacaactggtggatctgtacaaggtgctggagagcaggggctccgacccaaagccagaaaacccagcctgtccctggacggtgctcccagcaggtgaccttcccacccatgatggctacttaccctccaacatagatgacctcccctcacatgaggcacctctcgctgactctctggaagaactggagcctcagcacatctccctttctgttttcccctcaagttctcttcacccactcaccttctcctgtggtgataagctgactctggatcagttaaagatgaggtgtgactccctcatgctctga

SEQ ID NO: 3 - DNA, 1515 bp, Homo sapiens
  source 1..1515: mol_type = other DNA
atgggttggtcctgcatcatcctgtttctcgtggccaccgccaccggcgtgcactccgaaattgtgttgacacagtctccagccaccctgtctttgtctccaggggaaagagccaccctctcctgcagggccagtcagagtgttcgcagctacttagcctggtaccaacagaaacctggccaggctcccaggctcctcatctatgatgcatccaacagggccactggcatcccagccaggttcagtggcagtgggtctgggacagacttcactctcaccatcagcagcctagagcctgaagattttgcagtttattactgtcagcagcgtagcaactggcctccgacgttcggccaagggaccaaggtggaaatcaaaagtggagggggcggttcacagctgcaggtgcaggagtcgggcccaggactggtgaagccttcggagaccctgtccctcacctgcactgtctctggtggctccatcagcaacagttatttctcctggggctggatccgccagcccccagggaagggactggagtggattgggagtttctattatggtgaaaaaacctactacaacccgtccctcaagagccgagccaccatatccattgacacgtccaagagccagttctccctgaagctgagctctgtgaccgccgcagacacggctgtgtattactgtccgagagggcctactatgattcggggagttatagactcctggggccagggaaccctggtgacggtgtcgtcggggggcggggggagtcaggtgcagctggtgcagtccggagccgaggtaaagaagccaggcgcttccgtcaaggtgtcatgcaaggcctcaggctacaccttcacaagctattacatccactgggtgcgccaagctcccggtcagggcttggagtggatcgggtgcatttacccagggaacgtcaacacaaactacaacgagaagttcaaggatcgggcaaccctgaccgtggacacatccatctctaccgcctacatggagctgtcacgcctgcgctctgatgacaccgcagtgtacttctgtaccaggagtcactacggcctggactggaactttgatgtctggggccagggaaccaccgtgacggtgtccagtgtggagggcggtagtggcggctctggtgggtccggaggctcaggcggcgtgatggatgacattcagatgacccagagtccctcctccctctccgcttccgtcggagaccgcgtgaccatcacttgtcacgcctcacagaatatctacgtgtggctgaactggtaccaacagaagcccggcaaggcccccaagctgcttatctataaagcgtccaacctccacacgggagtcccttcccgcttctccggatccggcagtgggacggacttcacactcacaatctcgtcgctgcagccagaggactttgcgacgtactactgccagcagggccagacctacccatatactttcggcggcgggaccaaggtggagattaagtaa

SEQ ID NO: 4 - DNA, 1515 bp, Homo sapiens
  source 1..1515: mol_type = other DNA
atgggttggtcctgcatcatcctgtttctcgtggccaccgccaccggcgtgcactccgaaattgtgttgacacagtctccagccaccctgtctttgtctccaggggaaagagccaccctctcctgcagggccagtcagagtgttagaagtttcttagcctggtaccaacagaaacctggccaggctcccaggctcctcatctatgatgcatccaacagggccactggcatcccagccaggttcagtggcagtggggtctgggacagacttcactctcaccatcagcagcctagagcctgaagattttgcagtttattactgtcagcagcgtagcaactggcctccgacgttcggccaagggaccaaggtggaaatcaaaagtggagggggcggttcacagctacagctgcaggagtcgggcccaggactggtgaagccttcggagaccctatccctcacctgcactgtctctggtggctccatcagcagtagtagttactcctggggctggatccgccagcccccagggaagggcctggagtggattggagtttctattacagtgggatcacctactacagcccgtccctcaagagtcgaattatcatatccgaagacacgtccaagaaccagttctccctgaagctgagttctgtgaccgccgcagacacggctgtgtattactgtgcgagcgggtttactatgattcggggagcccttgactactggggccagggaaccctggtgacggtgtcgtcggggggcggggggagtcaggtgcagctggtgcagtccggagccgaggtaaagaagccaggcgcttccgtcaaggtgtcatgcaaggcctcaggctacaccttcacaagctattacatccactgggtgcgccaagctcccggtcagggcttggagtggatcgggtgcatttacccagggaacgtcaacacaaactacaacgagaagttcaaggatcgggcaaccctgaccgtggacacatccatctctaccgcctacatggagctgtcacgcctgcgctctgatgacaccgcagtgtacttctgtaccaggagtcactacggcctggactggaactttgatgtctggggccagggaaccaccgtgacggtgtccagtgtggagggcggtagtggcggctctggtgggtccggaggctcaggcggcgtgatggatgacattcagatgacccagagtccctcctccctctccgcttccgtcggagaccgcgtgaccatcacttgtcacgcctcacagaatatctacgtgtggctgaactggtaccaacagaagcccggcaaggcccccaagctgcttatctataaagcgtccaacctccacacgggagtcccttcccgcttctccggatccggcagtgggacggacttcacactcacaatctcgtcgctgcagccagaggactttgcgacgtactactgccagcagggccagacctacccatatactttcggcggcgggaccaaggtggagattaagtaa

SEQ ID NO: 5 - DNA, 1449 bp, Homo sapiens
  source 1..1449: mol_type = other DNA
atggatccccagtgcactatgggactgagtaacattctctttgtgatggccttcctgctctctggtgctgctcctctgaagattcaagcttatttcaatgagactgcagacctgccatgccaatttgcaaactctcaaaaccaaagcctgagtgagctagtagtattttggcaggaccaggaaaacttggttctgaatgaggtatacttaggcaaagagaaatttgacagtgttcattccaagtatatgggccgcacaagttttgattcggacagttggaccctgagacttcacaatcttcagatcaaggacaagggcttgtatcaatgtatcatccatcacaaaaagcccacaggaatgattcgcatccaccagatgaattctgaactgtcagtgcttgctaacttcagtcaacctgaaatagtaccaatttctaatataacagaaaatgtgtacataaatttgacctgctcatctatacacggttacccagaacctaagaagatgagtgttttgctaagaaccaagaattcaactatcgagtatgatggtattatgcagaaatctcaagataatgtcacagaactgtacgacgtttccatcagcttgtctgtttcattccctgatgttacgagcaatatgaccatcttctgtattctggaaactgacaagacgcggcttttatcttcacctttctctatagagcttgaggaccctcagcctcccccagaccacattcctggcggagggggaagtggcgggggtgggtccggcggcggcggctcgtttactgtcacggttcccaaggacctatatgtggtagagtatggtagcaatatgacaattgaatgcaaattcccagtagaaaaacaattagacctggctgcactaattgtctattgggaaatggaggataagaacattattcaatttgtgcatggagaggaagacctgaaggttcagcatagtagctacagacagagggcccggctgttgaaggaccagctctccctgggaaatgctgcacttcagatcacagatgtgaaattgcaggatgcaggggtgtaccgctgcatgatcagctatggtggtgccgactacaagcgaattactgtgaaagtcaatgccccatacaacaaaatcaaccaaagaattttggttgtggatccagtcacctctgaacatgaactgacatgtcaggctgagggctaccccaaggccgaagtcatctggacaagcagtgaccatcaagtcctgagtggtaagaccaccaccaccaattccaagagagaggagaagcttttcaatgtgaccagcacactgagaatcaacacaacaactaatgagattttctactgcacttttaggagattagatcctgaggaaaaccatacagctgaattggtcatcccagaactacctctggcacatcctccaaatgaaaggtaa

SEQ ID NO: 6 - DNA, 1392 bp, Homo sapiens
  source 1..1392: mol_type = other DNA
atggatccccagtgcactatgggactgagtaacattctctttgtgatggccttcctgctctctggtgctgctcctctgaagattcaagcttatttcaatgagactgcagacctgccatgccaatttgcaaactctcaaaaccaaagcctgagtgagctagtagtattttggcaggaccaggaaaacttggttctgaatgaggtatacttaggcaaagagaaatttgacagtgttcattccaagtatatgggccgcacaagttttgattcggacagttggaccctgagacttcacaatcttcagatcaaggacaagggcttgtatcaatgtatcatccatcacaaaaagcccacaggaatgattcgcatccaccagatgaattctgaactgtcagtgcttgctaacttcagtcaacctgaaatagtaccaatttctaatataacagaaaatgtgtacataaatttgacctgctcatctatacacggttacccagaacctaagaagatgagtgttttgctaagaaccaagaattcaactatcgagtatgatggtattatgcagaaatctcaagataatgtcacagaactgtacgacgtttccatcagcttgtctgtttcattccctgatgttacgagcaatatgaccatcttctgtattctggaaactgacaagacgcggcttttatcttcacctttctctatagagcttgaggaccctcagcctcccccagaccacattcctggcggagggggaagtggcgggggtgggtccggcggcggcggctcgttattcacagtgacagtccctaaggaactgtacataatagagcatggcagcaatgtgaccctggaatgcaactttgacactggaagtcatgtgaaccttggagcaataacagccagtttgcaaaaggtggaaaatgatacatccccacaccgtgaaagagccactttgctggaggagcagctgcccctagggaaggcctcgttccacatacctcaagtccaagtgagggacgaaggacagtaccaatgcataatcatctatggggtcgcctgggactacaagtacctgactctgaaagtcaaagcttcctacaggaaaataaacactcacatcctaaaggttccagaaacagatgaggtagagctcacctgccaggctacaggttatcctctggcagaagtatcctggccaaacgtcagcgttcctgccaacaccagccactccaggacccctgaaggcctctaccaggtcaccagtgttctgcgcctaaagccaccccctggcagaaacttcagctgtgtgttctggaatactcacgtgagggaacttactttggccagcattgaccttcaaagtcagatggaacccaggacccatccaacttaa

SEQ ID NO: 7 - DNA, 1434 bp, Homo sapiens
  source 1..1434: mol_type = other DNA
atgggccacacacggaggcagggaacatcaccatccaagtgtccatacctcaatttctttcagctcttggtgctggctggtctttctcacttctgttcaggtgttatccacgtgaccaaggaagtgaaagaagtggcaacgctgtcctgtggtcacaatgtttctgttgaagagctggcacaaactcgcatctactggcaaaaggagaagaaaatggtgctgactatgatgtctggggacatgaatatatggcccgagtacaagaaccggaccatctttgatatcactaataacctctccattgtgatcctggctctgcgcccatctgacgagggcacatacgagtgtgttgttctgaagtatgaaaaagacgctttcaagcgggaacacctggctgaagtgacgttatcagtcaaagctgacttccctacacctagtatatctgactttgaaattccaacttctaatattagaaggataatttgctcaacctctggaggttttccagagcctcacctctcctggttggaaaatggagaagaattaaatgccatcaacacaacagtttcccaagatcctgaaactgagctctatgctgttagcagcaaactggatttcaatatgacaaccaaccacagcttcatgtgtctcatcaagtatggacatttaagagtgaatcagaccttcaactggaatacaaccaagcaagagcattttcctgataacggcggagggggaagtggcgggggtgggtccggcggcggcggctcgtttactgtcacggttcccaaggacctatatgtggtagagtatggtagcaatatgacaattgaatgcaaattcccagtagaaaaacaattagacctggctgcactaattgtctattgggaaatggaggataagaacattattcaatttgtgcatggagaggaagacctgaaggttcagcatagtagctacagacagagggcccggctgttgaaggaccagctctccctgggaaatgctgcacttcagatcacagatgtgaaattgcaggatgcaggggtgtaccgctgcatgatcagctatggtggtgccgactacaagcgaattactgtgaaagtcaatgccccatacaacaaaatcaaccaaagaattttggttgtggatccagtcacctctgaacatgaactgacatgtcaggctgagggctaccccaaggccgaagtcatctggacaagcagtgaccatcaagtcctgagtggtaagaccaccaccaccaattccaagagagaggagaagcttttcaatgtgaccagcacactgagaatcaacacaacaactaatgagattttctactgcacttttaggagattagatcctgaggaaaaccatacagctgaattggtcatcccagaactacctctggcacatcctccaaatgaaaggtaa

SEQ ID NO: 8 - DNA, 1377 bp, Homo sapiens
  source 1..1377: mol_type = other DNA
atgggccacacacggaggcagggaacatcaccatccaagtgtccatacctcaatttctttcagctcttggtgctggctggtctttctcacttctgttcaggtgttatccacgtgaccaaggaagtgaaagaagtggcaacgctgtcctgtggtcacaatgtttctgttgaagagctggcacaaactcgcatctactggcaaaaggagaagaaaatggtgctgactatgatgtctggggacatgaatatatggcccgagtacaagaaccggaccatctttgatatcactaataacctctccattgtgatcctggctctgcgcccatctgacgagggcacatacgagtgtgttgttctgaagtatgaaaaagacgctttcaagcgggaacacctggctgaagtgacgttatcagtcaaagctgacttccctacacctagtatatctgactttgaaattccaacttctaatattagaaggataatttgctcaacctctggaggttttccagagcctcacctctcctggttggaaaatggagaagaattaaatgccatcaacacaacagtttcccaagatcctgaaactgagctctatgctgttagcagcaaactggatttcaatatgacaaccaaccacagcttcatgtgtctcatcaagtatggacatttaagagtgaatcagaccttcaactggaatacaaccaagcaagagcattttcctgataacggcggagggggaagtggcgggggtgggtccggcggcggcggctcgttattcacagtgacagtccctaaggaactgtacataatagagcatggcagcaatgtgaccctggaatgcaactttgacactggaagtcatgtgaaccttggagcaataacagccagtttgcaaaaggtggaaaatgatacatccccacaccgtgaaagagccactttgctggaggagcagctgcccctagggaaggcctcgttccacatacctcaagtccaagtgagggacgaaggacagtaccaatgcataatcatctatggggtcgcctgggactacaagtacctgactctgaaagtcaaagcttcctacaggaaaataaacactcacatcctaaaggttccagaaacagatgaggtagagctcacctgccaggctacaggttatcctctggcagaagtatcctggccaaacgtcagcgttcctgccaacaccagccactccaggacccctgaaggcctctaccaggtcaccagtgttctgcgcctaaagccaccccctggcagaaacttcagctgtgtgttctggaatactcacgtgagggaacttactttggccagcattgaccttcaaagtcagatggaacccaggacccatccaacttaa

SEQ ID NO: 9 - DNA, 1440 bp, Homo sapiens
  source 1..1440: mol_type = other DNA
atgaggatatttgctgtctttatattcatgacctactggcatttgctgaacgcatttactgtcacggttcccaaggacctatatgtggtagagtatggtagcaatatgacaattgaatgcaaattcccagtagaaaaacaattagacctggctgcactaattgtctattgggaaatggaggataagaacattattcaatttgtgcatggagaggaagacctgaaggttcagcatagtagctacagacagagggcccggctgttgaaggaccagctctccctgggaaatgctgcacttcagatcacagatgtgaaattgcaggatgcaggggtgtaccgctgcatgatcagctatggtggtgccgactacaagcgaattactgtgaaagtcaatgccccatacaacaaaatcaaccaaagaattttggttgtggatccagtcacctctgaacatgaactgacatgtcaggctgagggctaccccaaggccgaagtcatctggacaagcagtgaccatcaagtcctgagtggtaagaccaccaccaccaattccaagagagaggagaagcttttcaatgtgaccagcacactgagaatcaacacaacaactaatgagattttctactgcacttttaggagattagatcctgaggaaaaccatacagctgaattggtcatcccagaactacctctggcacatcctccaaatgaaaggggcggagggggaagtggcgggggtgggtccggcggcggcggctcgggtgctgctcctctgaagattcaagcttatttcaatgagactgcagacctgccatgccaatttgcaaactctcaaaaccaaagcctgagtgagctagtagtattttggcaggaccaggaaaacttggttctgaatgaggtatacttaggcaaagagaaatttgacagtgttcattccaagtatatgggccgcacaagttttgattcggacagttggaccctgagacttcacaatcttcagatcaaggacaagggcttgtatcaatgtatcatccatcacaaaaagcccacaggaatgattcgcatccaccagatgaattctgaactgtcagtgcttgctaacttcagtcaacctgaaatagtaccaatttctaatataacagaaaatgtgtacataaatttgacctgctcatctatacacggttacccagaacctaagaagatgagtgttttgctaagaaccaagaattcaactatcgagtatgatggtattatgcagaaatctcaagataatgtcacagaactgtacgacgtttccatcagcttgtctgtttcattccctgatgttacgagcaatatgaccatcttctgtattctggaaactgacaagacgcggcttttatcttcacctttctctatagagcttgaggaccctcagcctcccccagaccacattccttaa

SEQ ID NO: 10 - DNA, 1408 bp, Homo sapiens
  source 1..1408: mol_type = other DNA
atgaggatatttgctgtctttatattcatgacctactggcatttgctgaacgcatttactgtcacggttcccaaggacctatatgtggtagagtatggtagcaatatgacaattgaatgcaaattcccagtagaaaaacaattagacctggctgcactaattgtctattgggaaatggaggataagaacattattcaatttgtgcatggagaggaagacctgaaggttcagcatagtagctacagacagagggcccggctgttgaaggaccagctctccctgggaaatgctgcacttcagatcacagatgtgaaattgcaggatgcaggggtgtaccgctgcatgatcagctatggtggtgccgactacaagcgaattactgtgaaagtcaatgccccatacaacaaaatcaaccaaagaattttggttgtggatccagtcacctctgaacatgaactgacatgtcaggctgagggctaccccaaggccgaagtcatctggacaagcagtgaccatcaagtcctgagtggtaagaccaccaccaccaattccaagagagaggagaagcttttcaatgtgaccagcacactgagaatcaacacaacaactaatgagattttctactgcacttttaggagattagatcctgaggaaaaccatacagctgaattggtcatcccagaactacctctggcacatcctccaaatgaaaggggcggagggggaagtggcgggggtgggtccggcggcggcggctcgtctttctcacttctgttcaggtgttatccacgtgaccaaggaagtgaaagaagtggcaacgctgtcctgtggtcacaatgtttctgttgaagagctggcacaaactcgcatctactggcaaaaggagaagaaaatggtgctgactatgatgtctggggacatgaatatatggcccgagtacaagaaccggaccatctttgatatcactaataacctctccattgtgatcctggctctgcgcccatctgacgagggcacatacgagtgtgttgttctgaagtatgaaaaagacgctttcaagcgggaacacctggctgaagtgacgttatcagtcaaagctgacttccctacacctagtatatctgactttgaaattccaacttctaatattagaaggataatttgctcaacctctggaggttttccagagcctcacctctcctggttggaaaatggagaagaattaaatgccatcaacacaacagtttcccaagatcctgaaactgagctctatgctgttagcagcaaactggatttcaatatgacaaccaaccacagcttcatgtgtctcatcaagtatggacatttaagagtgaatcagaccttcaactggaatacaaccaagcaagagcattttcctgataactaa

SEQ ID NO: 11 - DNA, 1383 bp, Homo sapiens
  source 1..1383: mol_type = other DNA
atgatcttcctcctgctaatgttgagcctggaattgcagcttcaccagatagcagctttattcacagtgacagtccctaaggaactgtacataatagagcatggcagcaatgtgaccctggaatgcaactttgacactggaagtcatgtgaaccttggagcaataacagccagtttgcaaaaggtggaaaatgatacatccccacaccgtgaaagagccactttgctggaggagcagctgcccctagggaaggcctcgttccacatacctcaagtccaagtgagggacgaaggacagtaccaatgcataatcatctatggggtcgcctgggactacaagtacctgactctgaaagtcaaagcttcctacaggaaaataaacactcacatcctaaaggttccagaaacagatgaggtagagctcacctgccaggctacaggttatcctctggcagaagtatcctggccaaacgtcagcgttcctgccaacaccagccactccaggacccctgaaggcctctaccaggtcaccagtgttctgcgcctaaagccaccccctggcagaaacttcagctgtgtgttctggaatactcacgtgagggaacttactttggccagcattgaccttcaaagtcagatggaacccaggacccatccaactggcggagggggaagtggcgggggtgggtccggcggcggcggctcgggtgctgctcctctgaagattcaagcttatttcaatgagactgcagacctgccatgccaatttgcaaactctcaaaaccaaagcctgagtgagctagtagtattttggcaggaccaggaaaacttggttctgaatgaggtatacttaggcaaagagaaatttgacagtgttcattccaagtatatgggccgcacaagttttgattcggacagttggaccctgagacttcacaatcttcagatcaaggacaagggcttgtatcaatgtatcatccatcacaaaaagcccacaggaatgattcgcatccaccagatgaattctgaactgtcagtgcttgctaacttcagtcaacctgaaatagtaccaatttctaatataacagaaaatgtgtacataaatttgacctgctcatctatacacggttacccagaacctaagaagatgagtgttttgctaagaaccaagaattcaactatcgagtatgatggtattatgcagaaatctcaagataatgtcacagaactgtacgacgtttccatcagcttgtctgtttcattccctgatgttacgagcaatatgaccatcttctgtattctggaaactgacaagacgcggcttttatcttcacctttctctatagagcttgaggaccctcagcctcccccagaccacattcct

SEQ ID NO: 12 - protein, 254 aa, synthetic construct
  REGION 1..254: note = vector
MGWSCIILFLVATATGVHSEIVLTQSPATLSLSPGERATLSCRASQSVSSYLAWYQQKPGQAPRLLIYDASNRATGIPARFSGSGSGTDFTLTISSLEPEDFAVYYCQQRSNWPTFGQGTKVEIKSGGGGSQVQLVQSGAEVKKPGSSVKVSCKTSGDTFSTYAISWVRQAPGQGLEWMGGIIPIFGKAHYAQKFQGRVTITADESTSTAYMELSSLRSEDTAVYFCARKFHFVSGSPFGMDVWGQGTTVTVSS

SEQ ID NO: 13 - protein, 253 aa, synthetic construct
  REGION 1..253: note = vector
MGWSCIILFLVATATGVHSAIQLTQSPSSLSASVGDRVTITCRASQGISSALAWYQQKPGKAPKLLIYDASSLESGVPSRFSGSGSGTDFTLTISSLQPEDFATYYCQQFNSYPFTFGPGTKVDIKSGGGGSEVQLVESGGGLVQPGRSLRLSCAASGITFDDYGMHWVRQAPGKGLEWVSGISWNRGRIEYADSVKGRFTISRDNAKNSLYLQMNSLRAEDTALYYCAKGRFRYFDWFLDYWGQGTLVTVSS

SEQ ID NO: 14 - protein, 254 aa, synthetic construct
  REGION 1..254: note = vector
MGWSCIILFLVATATGVHSEIVLTQSPATLSLSPGERATLSCRASQSVSSYLAWYQQKPGQAPRLLIYDASNRATGIPARFSGSGSGTDFTLTISSLEPEDFAVYYCQQRSNWPTFGQGTKVEIKSGGGGSQVQLVQSGAEVKKPGSSVKVSCKTSGDTFSSYAISWVRQAPGQGLEWMGGIIPIFGRAHYAQKFQGRVTITADESTSTAYMELSSLRSEDTAVYFCARKFHFVSGSPFGMDVWGQGTTVTVSS

SEQ ID NO: 15 - protein, 250 aa, synthetic construct
  REGION 1..250: note = vector
MGWSCIILFLVATATGVHSDIQMTQSPSSLSASVGDRVTITCRASQGISSWLAWYQQKPEKAPKSLIYAASSLQSGVPSRFSGSGSGTDFTLTISSLQPEDFATYYCQQYNSYPYTFGQGTKLEIKSGGGGSQVQLVQSGAEVKKPGASVKVSCKASGYTFTSYDVHWVRQAPGQRLEWMGWLHADTGITKFSQKFQGRVTITRDTSASTAYMELSSLRSEDTAVYYCARERIQLWFDYWGQGTLVTVSS

SEQ ID NO: 16 - protein, 249 aa, synthetic construct
  REGION 1..249: note = vector
MGWSCIILFLVATATGVHSEIVLTQSPATLSLSPGERATLSCRASQSVSSYLVWYQQKPGQAPRLLIYDASNRATGIPARFSGSGSGTDFTLTISSLEPEDFAVYYCQQRSNWPRTFGQGTKVEIKSGGGGSQVQLVQSGAEVKKPGASVKVSCKASGYTFTDYGFSWVRQAPGQGLEWMGWITAYNGNTNYAQKLQGRVTMTTDTSTSTVYMELRSLRSDDTAVYYCARDYFYGMDVWGQGTTVTVSS

SEQ ID NO: 17 - protein, 250 aa, synthetic construct
  REGION 1..250: note = vector
GGGGSQVQLVQSGAEVKKPGASVKVSCKASGYTFTSYYIHWVRQAPGQGLEWIGCIYPGNVNTNYNEKFKDRATLTVDTSISTAYMELSRLRSDDTAVYFCTRSHYGLDWNFDVWGQGTTVTVSSVEGGSGGSGGSGGSGGVDDIQMTQSPSSLSASVGDRVTITCHASQNIYVWLNWYQQKPGKAPKLLIYKASNLHTGVPSRFSGSGSGTDFTLTISSLQPEDFATYYCQQGQTYPYTFGGGTKVEIK

SEQ ID NO: 18 - protein, 5 aa, synthetic construct
GGGGS